European Patent Application EP 4 169 531 A1, published April 26, 2023. Title: Drugs containing active sulfur compounds as the main component. Applicant: Bio-Xcelerator, Inc. Akaike, Takaaki. The sequence listing filed with the application follows.

SEQUENCE LISTING (2 sequences)

SEQ ID NO: 1 - DNA, 978 bp, SARS-CoV-2
tctttacgtgaagttcgtactattaaggttttcactactgtggacaacatcaatttacatacgcaagttgtcgatatgagcatgacctacggccaacagtttgggcctacctacctggatggtgcagacgttactaagataaaacctcataattcgcacgagggcaaaaccttctatgttctgcccaacgatgataccctgcgtgtcgaagcattcgagtattatcacacgacggatccctcttttttgggtcgctacatgagtgctttgaaccacacaaagaaatggaagtacccgcaagtaaatggtttaaccagtattaagtgggcagacaacaactgttacctggcaactgcacttttaacgttacaacaaattgaactgaaattcaatccacctgcccttcaggacgcgtactaccgcgcacgggccggtgaggccgctaacttttgtgccctgattctggcgtactgtaataagaccgttggtgagcttggtgatgttcgtgaaactatgagttatttatttcagcatgccaatctggatagctgtaaaagagtacttaatgtggtctgtaaaacttgtggccagcaacagacgacgctgaaaggtgtagaggctgtcatgtatatgggcaccctgtcttatgagcagtttaaaaaaggagtacagattccgtgcacatgcggaaagcaggcgacgaaatatctggtgcagcaggaatcaccgtttgtgatgatgtccgctccaccggcgcagtatgaacttaaacatggaacctttacgtgcgcgtcagaatataccggcaattatcagtgcggccattataaacatattacctccaaagaaacattgtattgcatagatggggctctgttgaccaaaagctcagaatataaaggaccgatcacagatgtgttttataaagaaaattcgtatacaacaacaatcaaaccagtgacatataaactggacggg

SEQ ID NO: 2 - DNA, 918 bp, SARS CoV 2
tctggtttccgtaaaatggcgtttccctctggaaaggttgagggctgtatggtgcaagttacgtgtgggactaccacattgaacggtctttggctggatgatgttgtttactgtcctcgtcacgtgatttgcactagtgaggacatgttaaacccaaactacgaagatctgctgatacgtaaaagcaaccacaatttccttgtgcaagcaggtaacgttcagctgcgggtaattggtcattctatgcagaattgcgtgctgaagttaaaggttgacacggcaaaccctaaaacccccaaatataaattcgtgcgtattcaaccaggtcagacatttagtgttcttgcatgttacaacggttcaccgagtggtgtctatcagtgcgcaatgcggccgaatttcactattaaaggttcattcctgaatgggagctgtggctcagtcggtttcaatatcgattatgactgcgtatcgttttgctatatgcatcatatggaattgccgaccggcgttcacgccggcacagatctggaaggcaacttttatggaccgtttgtagaccgccagaccgcccaggcagctgggacagatacaacaattacggtcaacgttttggcctggctgtacgctgccgtgattaatggggaccgctggtttctgaatcgctttaccactacgctgaatgactttaatttggtggctatgaaatataattatgagcctctgacgcaggatcatgtggatatactgggcccgttgtccgctcaaaccggaatcgcggtcctggatatgtgtgcgtccttaaaagaacttcttcaaaatggcatgaatggaagaaccatcttaggaagcgcgttattagaagatgaatttactccatttgatgtcgtaagacagtgctcgggcgtaacctttcag